European Patent Application EP 4 678 732 A1, published January 14, 2026. Title: 分离的克里斯滕森菌、包含其的组合物及用途. Applicant: 慕恩（广州）生物科技有限公司. Application WO. The sequence listing filed with the application follows.

SEQUENCE LISTING (5 sequences)

SEQ ID NO: 1 - RNA, 1431 nt, Christensenella sp.
  source 1..1431: mol_type = rRNA
agatgcgaagcatcgagcaacacgcgaaaaaaagagctaacacgaggaaggaaagaagtgagtattgggtgcagaccgctagaccgagtggcggacgggtgagtaacgcgtgagcaacctgccctgcaacgggggacaacagttggaaacgactgctaataccgcataagaccacggtaccgcatggtacaggggtaaaaggatttattcgatgcaggatgggctcgcgtcccattagatagttggtgaggtaacggcccaccaagtcaacgatgggtagccgacctgagagggtgatcggccacactggaactgagacacggtccagactcctacgggaggcagcagtggggaatattgggcaatgggggaaaccctgacccagcaacgccgcgtgagggaagaaggtcttcggattgtaaacctttgtcctatgggacgaaacaaatgacggtaccataggaggaagctccggctaactacgtgccagcagccgcggtaatacgtagggagcaagcgttgtccggaattactgggcgtaaagggtgcgtaggtggtcatgtaagtcagatgtgaaagaccggggcttaaccccgggattgcatttgaaactgtgtgacttgagtacaggagagggaagtggaattcctagtgtagcggtgaaatgcgtagatattaggaggaacaccagtggcgaaggcgactttctggactgtaactgacactgaagcacgaaagcgtggggagcaaacaggattagataccctggtagtccacgccgtaaacgatggatactaggtgtggggcccgatagggttccgtgccgaagctaacgcattaagtatcccgcctggggagtacgatcgcaaggttgaaactcaaaggaattgacgggggcccgcacaagcagcggagcatgtggtttaattcgaagcaacgcgaagaaccttaccaaggcttgacatcgtctgacgactgtagagatacagtttcccttcggggcagacagacaggtggtgcatggttgtcgtcagctcgtgtcgtgagatgttgggttaagtcccgcaacgagcgcaacccttattgctagttgccagcacgtaaaggtgggaactctagtgagactgccggggacaactcggaggaaggtggggacgacgtcaaatcatcatgccccttatgtcttgggctacacacgtgctacaatggccggtacaaagggcagcgaacccgcaaggggaagcgaatctcaaaaagccggtcccagttcggattgtgggctgcaacccgcccacatgaagtcggagttgctagtaatcgcgaatcagcatgtcgcggtgaatgcgttcccgggccttgtacacaccgcccgtcacaccacggaagttgggagcacccgaagccagtggcttaaccgtaaggagagagctt

SEQ ID NO: 2 - RNA, 1477 nt, Christensenella sp.
  source 1..1477: mol_type = rRNA
tcgaacgagggtcatacgcgtgaactgcaccgagtacttacgaaagaccggagtgaaagcgaagcgtttttgcgagatgcgaagcatcgagcaacacgcgaaaaaaagagctaacacgaggaaggaaagaagtgagtattgggtgcagaccgctagaccgagtggcggacgggtgagtaacgcgtgagcaacctgccctgcaacgggggacaacagttggaaacgactgctaataccgcataagaccacggtaccgcatggtacaggggtaaaaggatttattcgatgcaggatgggctcgcgtcccattagatagttggtgaggtaacggcccaccaagtcaacgatgggtagccgacctgagagggtgatcggccacactggaactgagacacggtccagactcctacgggaggcagcagtggggaatattgggcaatgggggaaaccctgacccagcaacgccgcgtgagggaagaaggtcttcggattgtaaacctttgtcctatgggacgaaacaaatgacggtaccataggaggaagctccggctaactacgtgccagcagccgcggtaatacgtagggagcaagcgttgtccggaattactgggcgtaaagggtgcgtaggtggtcatgtaagtcagatgtgaaagaccggggcttaaccccgggattgcatttgaaactgtgtgacttgagtacaggagagggaagtggaattcctagtgtagcggtgaaatgcgtagatattaggaggaacaccagtggcgaaggcgactttctggactgtaactgacactgaagcacgaaagcgtggggagcaaacaggattagataccctggtagtccacgccgtaaacgatggatactaggtgtggggcccgatagggttccgtgccgaagctaacgcattaagtatcccgcctggggagtacgatcgcaaggttgaaactcaaaggaattgacgggggcccgcacaagcagcggagcatgtggtttaattcgaagcaacgcgaagaaccttaccaaggcttgacatcgtctgacgactgtagagatacagtttcccttcggggcagacagacaggtggtgcatggttgtcgtcagctcgtgtcgtgagatgttgggttaagtcccgcaacgagcgcaacccttattgctagttgccagcacgtaaaggtgggaactctagtgagactgccggggacaactcggaggaaggtggggacgacgtcaaatcatcatgccccttatgtcttgggctacacacgtgctacaatggccggtacaaagggcagcgaacccgcaaggggaagcgaatctcaaaaagccggtcccagttcggattgtgggctgcaacccgcccacatgaagtcggagttgctagtaatcgcgaatcagcatgtcgcggtgaatgcgttcccgggccttgtacacaccgcccgtcacaccacggaagttgggagcacccgaagc

SEQ ID NO: 3 - RNA, 1376 nt, Christensenella sp.
  source 1..1376: mol_type = rRNA
tcgaacgaagttgctctttgtgaagccctcgggtggaactgcgagtatacttagtggcggacgggtgagtaacgcgtgagcaatctgccctgcaatgggggacaacagttggaaacgactgctaataccgcatgagaccacgaaaccgcatggttttgaggtaaaaggatttattcgatgcaggatgagctcgcgtcccattagatagttggtgaggtaacggcccaccaagtcaacgatgggtagccgacctgagagggtgatcggccacactggaactgagacacggtccagactcctacgggaggcagcagtggggaatattgggcaatgggggaaaccctgacccagcaacgccgcgtgagggaagaaggtcttcggattgtaaacctttgtcctatgggacgaaacaaatgacggtaccataggaggaagctccggctaactacgtgccagcagccgcggtaatacgtagggagcaagcgttgtccggaattactgggcgtaaagggtgcgtaggtggctatgtaagtcagatgtgaaagaccggggcttaaccccggggttgcatttgaaactgtgtggcttgagtacaggagagggaagtggaattcctagtgtagcggtgaaatgcgtagatattaggaggaacaccagtggcgaaggcgactttctggactgtaactgacactgaagcacgaaagcgtggggagcaaacaggattagataccctggtagtccacgccgtaaacgatggatactaggtgtggggcccgatagggttccgtgccgaagctaacgcattaagtatcccgcctggggagtacgatcgcaaggttgaaactcaaaggaattgacgggggcccgcacaagcagcggagcatgtggtttaattcgaagcaacgcgaagaaccttaccaaggcttgacatcctctgacgactgtagagatacagtttcccttcggggcagagagacaggtggtgcatggttgtcgtcagctcgtgtcgtgagatgttgggttaagtcccgcaacgagcgcaacccttattgctagttgccagcgcgtaaaggcgggaactctagtgagactgccggggacaactcggaggaaggtggggacgacgtcaaatcatcatgccccttatgtcttgggctacacacgtgctacaatggccggtacaaagggcagcgaacccgtaaggggaagcgaatctcaaaaagccggtcccagttcggattgtgggctgcaacccgcccacatgaagtcggagttgctagtaatcgcgaatcagcatgtcgcggtgaatgcgttcccgggccttgtacacaccgcccgtcacaccacggaagttgggagcacccgaagccagtagg

SEQ ID NO: 4 - DNA, 20 bp, synthetic construct
  source 1..20: mol_type = other DNA
agagtttgatcmtggctcag

SEQ ID NO: 5 - DNA, 22 bp, synthetic construct
  source 1..22: mol_type = other DNA
tacggytaccttgttacgactt